European Patent Application EP 4 296 673 A2, published December 27, 2023. Title: PEPTIDES AND METHODS FOR THE DETECTION OF LYME DISEASE ANTIBODIES. Applicant: ZOETIS SERVICES LLC. Application US. The sequence listing filed with the application follows.

SEQUENCE LISTING (152 sequences)

SEQ ID NO: 1 - protein, 25 aa, Borrelia sp.
  VARIANT 11: note = V or L
  VARIANT 16: note = L or I
  VARIANT 17: note = A or V
  VARIANT 21: note = R, D or N
  VARIANT 24: note = I, W or Y
  VARIANT 25: note = K or R
LKKDDNIAAAXVLRGXXKDGXFAXX

SEQ ID NO: 2 - protein, 48 aa, Borrelia sp.
  VARIANT 1: note = A or V
  VARIANT 2: note = E or D
  VARIANT 5: note = K or R
  VARIANT 6: note = K or R
  VARIANT 18: note = V or L
  VARIANT 23: note = L or I
  VARIANT 24: note = A or V
  VARIANT 28: note = R, D or N
  VARIANT 31: note = I, W or Y
  VARIANT 32: note = K or R
  VARIANT 35: note = Q or R
  VARIANT 38: note = V or A
XXSPXXPLKKDDNIAAAXVLRGXXKDGXFAXXAVXEGXQQEGAQQPSC

SEQ ID NO: 3 - protein, 25 aa, Borrelia sp.
LKKDDNIAAAVVLRGLAKDGRFAIK

SEQ ID NO: 4 - protein, 25 aa, Borrelia sp.
LKKDDNIAAALVLRGLAKDGRFAIK

SEQ ID NO: 5 - protein, 25 aa, Borrelia sp.
LKKDDNIAAAVVLRGIAKDGRFAIK

SEQ ID NO: 6 - protein, 25 aa, Borrelia sp.
LKKDDNIAAALVLRGIAKDGRFAIK

SEQ ID NO: 7 - protein, 25 aa, Borrelia sp.
LKKDDNIAAAVVLRGLVKDGRFAIK

SEQ ID NO: 8 - protein, 25 aa, Borrelia sp.
LKKDDNIAAALVLRGLVKDGRFAIK

SEQ ID NO: 9 - protein, 25 aa, Borrelia sp.
LKKDDNIAAAVVLRGIVKDGRFAIK

SEQ ID NO: 10 - protein, 25 aa, Borrelia sp.
LKKDDNIAAALVLRGIVKDGRFAIK

SEQ ID NO: 11 - protein, 25 aa, Borrelia sp.
LKKDDNIAAAVVLRGLAKDGDFAIK

SEQ ID NO: 12 - protein, 25 aa, Borrelia sp.
LKKDDNIAAALVLRGLAKDGDFAIK

SEQ ID NO: 13 - protein, 25 aa, Borrelia sp.
LKKDDNIAAAVVLRGIAKDGDFAIK

SEQ ID NO: 14 - protein, 25 aa, Borrelia sp.
LKKDDNIAAALVLRGIAKDGDFAIK

SEQ ID NO: 15 - protein, 25 aa, Borrelia sp.
LKKDDNIAAAVVLRGLVKDGDFAIK

SEQ ID NO: 16 - protein, 25 aa, Borrelia sp.
LKKDDNIAAALVLRGLVKDGDFAIK

SEQ ID NO: 17 - protein, 25 aa, Borrelia sp.
LKKDDNIAAAVVLRGIVKDGDFAIK

SEQ ID NO: 18 - protein, 25 aa, Borrelia sp.
LKKDDNIAAALVLRGIVKDGDFAIK

SEQ ID NO: 19 - protein, 25 aa, Borrelia sp.
LKKDDNIAAAVVLRGLAKDGNFAIK

SEQ ID NO: 20 - protein, 25 aa, Borrelia sp.
LKKDDNIAAALVLRGLAKDGNFAIK

SEQ ID NO: 21 - protein, 25 aa, Borrelia sp.
LKKDDNIAAAVVLRGIAKDGNFAIK

SEQ ID NO: 22 - protein, 25 aa, Borrelia sp.
LKKDDNIAAALVLRGIAKDGNFAIK

SEQ ID NO: 23 - protein, 25 aa, Borrelia sp.
LKKDDNIAAAVVLRGLVKDGNFAIK

SEQ ID NO: 24 - protein, 25 aa, Borrelia sp.
LKKDDNIAAALVLRGLVKDGNFAIK

SEQ ID NO: 25 - protein, 25 aa, Borrelia sp.
LKKDDNIAAAVVLRGIVKDGNFAIK

SEQ ID NO: 26 - protein, 25 aa, Borrelia sp.
LKKDDNIAAALVLRGIVKDGNFAIK

SEQ ID NO: 27 - protein, 25 aa, Borrelia sp.
LKKDDNIAAAVVLRGLAKDGRFAWK

SEQ ID NO: 28 - protein, 25 aa, Borrelia sp.
LKKDDNIAAALVLRGLAKDGRFAWK

SEQ ID NO: 29 - protein, 25 aa, Borrelia sp.
LKKDDNIAAAVVLRGIAKDGRFAWK

SEQ ID NO: 30 - protein, 25 aa, Borrelia sp.
LKKDDNIAAALVLRGIAKDGRFAWK

SEQ ID NO: 31 - protein, 25 aa, Borrelia sp.
LKKDDNIAAAVVLRGLVKDGRFAWK

SEQ ID NO: 32 - protein, 25 aa, Borrelia sp.
LKKDDNIAAALVLRGLVKDGRFAWK

SEQ ID NO: 33 - protein, 25 aa, Borrelia sp.
LKKDDNIAAAVVLRGIVKDGRFAWK

SEQ ID NO: 34 - protein, 25 aa, Borrelia sp.
LKKDDNIAAALVLRGIVKDGRFAWK

SEQ ID NO: 35 - protein, 25 aa, Borrelia sp.
LKKDDNIAAAVVLRGLAKDGDFAWK

SEQ ID NO: 36 - protein, 25 aa, Borrelia sp.
LKKDDNIAAALVLRGLAKDGDFAWK

SEQ ID NO: 37 - protein, 25 aa, Borrelia sp.
LKKDDNIAAAVVLRGIAKDGDFAWK

SEQ ID NO: 38 - protein, 25 aa, Borrelia sp.
LKKDDNIAAALVLRGIAKDGDFAWK

SEQ ID NO: 39 - protein, 25 aa, Borrelia sp.
LKKDDNIAAAVVLRGLVKDGDFAWK

SEQ ID NO: 40 - protein, 25 aa, Borrelia sp.
LKKDDNIAAALVLRGLVKDGDFAWK

SEQ ID NO: 41 - protein, 25 aa, Borrelia sp.
LKKDDNIAAAVVLRGIVKDGDFAWK

SEQ ID NO: 42 - protein, 25 aa, Borrelia sp.
LKKDDNIAAALVLRGIVKDGDFAWK

SEQ ID NO: 43 - protein, 25 aa, Borrelia sp.
LKKDDNIAAAVVLRGLAKDGNFAWK

SEQ ID NO: 44 - protein, 25 aa, Borrelia sp.
LKKDDNIAAALVLRGLAKDGNFAWK

SEQ ID NO: 45 - protein, 25 aa, Borrelia sp.
LKKDDNIAAAVVLRGIAKDGNFAWK

SEQ ID NO: 46 - protein, 25 aa, Borrelia sp.
LKKDDNIAAALVLRGIAKDGNFAWK

SEQ ID NO: 47 - protein, 25 aa, Borrelia sp.
LKKDDNIAAAVVLRGLVKDGNFAWK

SEQ ID NO: 48 - protein, 25 aa, Borrelia sp.
LKKDDNIAAALVLRGLVKDGNFAWK

SEQ ID NO: 49 - protein, 25 aa, Borrelia sp.
LKKDDNIAAAVVLRGIVKDGNFAWK

SEQ ID NO: 50 - protein, 25 aa, Borrelia sp.
LKKDDNIAAALVLRGIVKDGNFAWK

SEQ ID NO: 51 - protein, 25 aa, Borrelia sp.
LKKDDNIAAAVVLRGLAKDGRFAYK

SEQ ID NO: 52 - protein, 25 aa, Borrelia sp.
LKKDDNIAAALVLRGLAKDGRFAYK

SEQ ID NO: 53 - protein, 25 aa, Borrelia sp.
LKKDDNIAAAVVLRGIAKDGRFAYK

SEQ ID NO: 54 - protein, 25 aa, Borrelia sp.
LKKDDNIAAALVLRGIAKDGRFAYK

SEQ ID NO: 55 - protein, 25 aa, Borrelia sp.
LKKDDNIAAAVVLRGLVKDGRFAYK

SEQ ID NO: 56 - protein, 25 aa, Borrelia sp.
LKKDDNIAAALVLRGLVKDGRFAYK

SEQ ID NO: 57 - protein, 25 aa, Borrelia sp.
LKKDDNIAAAVVLRGIVKDGRFAYK

SEQ ID NO: 58 - protein, 25 aa, Borrelia sp.
LKKDDNIAAALVLRGIVKDGRFAYK

SEQ ID NO: 59 - protein, 25 aa, Borrelia sp.
LKKDDNIAAAVVLRGLAKDGDFAYK

SEQ ID NO: 60 - protein, 25 aa, Borrelia sp.
LKKDDNIAAALVLRGLAKDGDFAYK

SEQ ID NO: 61 - protein, 25 aa, Borrelia sp.
LKKDDNIAAAVVLRGIAKDGDFAYK

SEQ ID NO: 62 - protein, 25 aa, Borrelia sp.
LKKDDNIAAALVLRGIAKDGDFAYK

SEQ ID NO: 63 - protein, 25 aa, Borrelia sp.
LKKDDNIAAAVVLRGLVKDGDFAYK

SEQ ID NO: 64 - protein, 25 aa, Borrelia sp.
LKKDDNIAAALVLRGLVKDGDFAYK

SEQ ID NO: 65 - protein, 25 aa, Borrelia sp.
LKKDDNIAAAVVLRGIVKDGDFAYK

SEQ ID NO: 66 - protein, 25 aa, Borrelia sp.
LKKDDNIAAALVLRGIVKDGDFAYK

SEQ ID NO: 67 - protein, 25 aa, Borrelia sp.
LKKDDNIAAAVVLRGLAKDGNFAYK

SEQ ID NO: 68 - protein, 25 aa, Borrelia sp.
LKKDDNIAAALVLRGLAKDGNFAYK

SEQ ID NO: 69 - protein, 25 aa, Borrelia sp.
LKKDDNIAAAVVLRGIAKDGNFAYK

SEQ ID NO: 70 - protein, 25 aa, Borrelia sp.
LKKDDNIAAALVLRGIAKDGNFAYK

SEQ ID NO: 71 - protein, 25 aa, Borrelia sp.
LKKDDNIAAAVVLRGLVKDGNFAYK

SEQ ID NO: 72 - protein, 25 aa, Borrelia sp.
LKKDDNIAAALVLRGLVKDGNFAYK

SEQ ID NO: 73 - protein, 25 aa, Borrelia sp.
LKKDDNIAAAVVLRGIVKDGNFAYK

SEQ ID NO: 74 - protein, 25 aa, Borrelia sp.
LKKDDNIAAALVLRGIVKDGNFAYK

SEQ ID NO: 75 - protein, 25 aa, Borrelia sp.
LKKDDNIAAAVVLRGLAKDGRFAIR

SEQ ID NO: 76 - protein, 25 aa, Borrelia sp.
LKKDDNIAAALVLRGLAKDGRFAIR

SEQ ID NO: 77 - protein, 25 aa, Borrelia sp.
LKKDDNIAAAVVLRGIAKDGRFAIR

SEQ ID NO: 78 - protein, 25 aa, Borrelia sp.
LKKDDNIAAALVLRGIAKDGRFAIR

SEQ ID NO: 79 - protein, 25 aa, Borrelia sp.
LKKDDNIAAAVVLRGLVKDGRFAIR

SEQ ID NO: 80 - protein, 25 aa, Borrelia sp.
LKKDDNIAAALVLRGLVKDGRFAIR

SEQ ID NO: 81 - protein, 25 aa, Borrelia sp.
LKKDDNIAAAVVLRGIVKDGRFAIR

SEQ ID NO: 82 - protein, 25 aa, Borrelia sp.
LKKDDNIAAALVLRGIVKDGRFAIR

SEQ ID NO: 83 - protein, 25 aa, Borrelia sp.
LKKDDNIAAAVVLRGLAKDGDFAIR

SEQ ID NO: 84 - protein, 25 aa, Borrelia sp.
LKKDDNIAAALVLRGLAKDGDFAIR

SEQ ID NO: 85 - protein, 25 aa, Borrelia sp.
LKKDDNIAAAVVLRGIAKDGDFAIR

SEQ ID NO: 86 - protein, 25 aa, Borrelia sp.
LKKDDNIAAALVLRGIAKDGDFAIR

SEQ ID NO: 87 - protein, 25 aa, Borrelia sp.
LKKDDNIAAAVVLRGLVKDGDFAIR

SEQ ID NO: 88 - protein, 25 aa, Borrelia sp.
LKKDDNIAAALVLRGLVKDGDFAIR

SEQ ID NO: 89 - protein, 25 aa, Borrelia sp.
LKKDDNIAAAVVLRGIVKDGDFAIR

SEQ ID NO: 90 - protein, 25 aa, Borrelia sp.
LKKDDNIAAALVLRGIVKDGDFAIR

SEQ ID NO: 91 - protein, 25 aa, Borrelia sp.
LKKDDNIAAAVVLRGLAKDGNFAIR

SEQ ID NO: 92 - protein, 25 aa, Borrelia sp.
LKKDDNIAAALVLRGLAKDGNFAIR

SEQ ID NO: 93 - protein, 25 aa, Borrelia sp.
LKKDDNIAAAVVLRGIAKDGNFAIR

SEQ ID NO: 94 - protein, 25 aa, Borrelia sp.
LKKDDNIAAALVLRGIAKDGNFAIR

SEQ ID NO: 95 - protein, 25 aa, Borrelia sp.
LKKDDNIAAAVVLRGLVKDGNFAIR

SEQ ID NO: 96 - protein, 25 aa, Borrelia sp.
LKKDDNIAAALVLRGLVKDGNFAIR

SEQ ID NO: 97 - protein, 25 aa, Borrelia sp.
LKKDDNIAAAVVLRGIVKDGNFAIR

SEQ ID NO: 98 - protein, 25 aa, Borrelia sp.
LKKDDNIAAALVLRGIVKDGNFAIR

SEQ ID NO: 99 - protein, 25 aa, Borrelia sp.
LKKDDNIAAAVVLRGLAKDGRFAWR

SEQ ID NO: 100 - protein, 25 aa, Borrelia sp.
LKKDDNIAAALVLRGLAKDGRFAWR

SEQ ID NO: 101 - protein, 25 aa, Borrelia sp.
LKKDDNIAAAVVLRGIAKDGRFAWR

SEQ ID NO: 102 - protein, 25 aa, Borrelia sp.
LKKDDNIAAALVLRGIAKDGRFAWR

SEQ ID NO: 103 - protein, 25 aa, Borrelia sp.
LKKDDNIAAAVVLRGLVKDGRFAWR

SEQ ID NO: 104 - protein, 25 aa, Borrelia sp.
LKKDDNIAAALVLRGLVKDGRFAWR

SEQ ID NO: 105 - protein, 25 aa, Borrelia sp.
LKKDDNIAAAVVLRGIVKDGRFAWR

SEQ ID NO: 106 - protein, 25 aa, Borrelia sp.
LKKDDNIAAALVLRGIVKDGRFAWR

SEQ ID NO: 107 - protein, 25 aa, Borrelia sp.
LKKDDNIAAAVVLRGLAKDGDFAWR

SEQ ID NO: 108 - protein, 25 aa, Borrelia sp.
LKKDDNIAAALVLRGLAKDGDFAWR

SEQ ID NO: 109 - protein, 25 aa, Borrelia sp.
LKKDDNIAAAVVLRGIAKDGDFAWR

SEQ ID NO: 110 - protein, 25 aa, Borrelia sp.
LKKDDNIAAALVLRGIAKDGDFAWR

SEQ ID NO: 111 - protein, 25 aa, Borrelia sp.
LKKDDNIAAAVVLRGLVKDGDFAWR

SEQ ID NO: 112 - protein, 25 aa, Borrelia sp.
LKKDDNIAAALVLRGLVKDGDFAWR

SEQ ID NO: 113 - protein, 25 aa, Borrelia sp.
LKKDDNIAAAVVLRGIVKDGDFAWR

SEQ ID NO: 114 - protein, 25 aa, Borrelia sp.
LKKDDNIAAALVLRGIVKDGDFAWR

SEQ ID NO: 115 - protein, 25 aa, Borrelia sp.
LKKDDNIAAAVVLRGLAKDGNFAWR

SEQ ID NO: 116 - protein, 25 aa, Borrelia sp.
LKKDDNIAAALVLRGLAKDGNFAWR

SEQ ID NO: 117 - protein, 25 aa, Borrelia sp.
LKKDDNIAAAVVLRGIAKDGNFAWR

SEQ ID NO: 118 - protein, 25 aa, Borrelia sp.
LKKDDNIAAALVLRGIAKDGNFAWR

SEQ ID NO: 119 - protein, 25 aa, Borrelia sp.
LKKDDNIAAAVVLRGLVKDGNFAWR

SEQ ID NO: 120 - protein, 25 aa, Borrelia sp.
LKKDDNIAAALVLRGLVKDGNFAWR

SEQ ID NO: 121 - protein, 25 aa, Borrelia sp.
LKKDDNIAAAVVLRGIVKDGNFAWR

SEQ ID NO: 122 - protein, 25 aa, Borrelia sp.
LKKDDNIAAALVLRGIVKDGNFAWR

SEQ ID NO: 123 - protein, 25 aa, Borrelia sp.
LKKDDNIAAAVVLRGLAKDGRFAYR

SEQ ID NO: 124 - protein, 25 aa, Borrelia sp.
LKKDDNIAAALVLRGLAKDGRFAYR

SEQ ID NO: 125 - protein, 25 aa, Borrelia sp.
LKKDDNIAAAVVLRGIAKDGRFAYR

SEQ ID NO: 126 - protein, 25 aa, Borrelia sp.
LKKDDNIAAALVLRGIAKDGRFAYR

SEQ ID NO: 127 - protein, 25 aa, Borrelia sp.
LKKDDNIAAAVVLRGLVKDGRFAYR

SEQ ID NO: 128 - protein, 25 aa, Borrelia sp.
LKKDDNIAAALVLRGLVKDGRFAYR

SEQ ID NO: 129 - protein, 25 aa, Borrelia sp.
LKKDDNIAAAVVLRGIVKDGRFAYR

SEQ ID NO: 130 - protein, 25 aa, Borrelia sp.
LKKDDNIAAALVLRGIVKDGRFAYR

SEQ ID NO: 131 - protein, 25 aa, Borrelia sp.
LKKDDNIAAAVVLRGLAKDGDFAYR

SEQ ID NO: 132 - protein, 25 aa, Borrelia sp.
LKKDDNIAAALVLRGLAKDGDFAYR

SEQ ID NO: 133 - protein, 25 aa, Borrelia sp.
LKKDDNIAAAVVLRGIAKDGDFAYR

SEQ ID NO: 134 - protein, 25 aa, Borrelia sp.
LKKDDNIAAALVLRGIAKDGDFAYR

SEQ ID NO: 135 - protein, 25 aa, Borrelia sp.
LKKDDNIAAAVVLRGLVKDGDFAYR

SEQ ID NO: 136 - protein, 25 aa, Borrelia sp.
LKKDDNIAAALVLRGLVKDGDFAYR

SEQ ID NO: 137 - protein, 25 aa, Borrelia sp.
LKKDDNIAAAVVLRGIVKDGDFAYR

SEQ ID NO: 138 - protein, 25 aa, Borrelia sp.
LKKDDNIAAALVLRGIVKDGDFAYR

SEQ ID NO: 139 - protein, 25 aa, Borrelia sp.
LKKDDNIAAAVVLRGLAKDGNFAYR

SEQ ID NO: 140 - protein, 25 aa, Borrelia sp.
LKKDDNIAAALVLRGLAKDGNFAYR

SEQ ID NO: 141 - protein, 25 aa, Borrelia sp.
LKKDDNIAAAVVLRGIAKDGNFAYR

SEQ ID NO: 142 - protein, 25 aa, Borrelia sp.
LKKDDNIAAALVLRGIAKDGNFAYR

SEQ ID NO: 143 - protein, 25 aa, Borrelia sp.
LKKDDNIAAAVVLRGLVKDGNFAYR

SEQ ID NO: 144 - protein, 25 aa, Borrelia sp.
LKKDDNIAAALVLRGLVKDGNFAYR

SEQ ID NO: 145 - protein, 25 aa, Borrelia sp.
LKKDDNIAAAVVLRGIVKDGNFAYR

SEQ ID NO: 146 - protein, 25 aa, Borrelia sp.
LKKDDNIAAALVLRGIVKDGNFAYR

SEQ ID NO: 147 - protein, 10 aa, Borrelia sp.
PVVAESPKKP

SEQ ID NO: 148 - protein, 14 aa, Borrelia sp.
ILMTLFLFISCNNS

SEQ ID NO: 149 - skipped

SEQ ID NO: 150 - protein, 15 aa, Borrelia sp.
  VARIANT 2: note = Q or R
  VARIANT 5: note = V or A
VXEGXQQEGAQQPSC

SEQ ID NO: 151 - protein, 16 aa, Borrelia sp.
  VARIANT 3: note = Q or R
  VARIANT 6: note = V or A
AVXEGXQQEGAQQPSC

SEQ ID NO: 152 - protein, 6 aa, synthetic construct
  REGION 1..6: note = 6X His tag
HHHHHH